European Patent Application EP 4 592 393 A1, published July 30, 2025. Title: Lipase variant. Applicant: 花王株式会社. The sequence listing filed with the application follows.

SEQUENCE LISTING (34 sequences)

SEQ ID NO: 1 - DNA, 882 bp, Serratia sp.
  source 1..882: mol_type = genomic DNA
atgtctacaacaacgaaattaaaatatccaatcattttagttcatggattcagcggatttgataaagttgccgggatttatccttatttttatggcattgaacaagcgcttgaaaaggcaggcgcgactgtgtttacggcagcaatatcggctgaaaatgccaatgaagtgaggggtgaacagctgctgaaatttgtgcagcaggtcatttcagtcaccggtgctgaaaaagtaaacctgatcggccactcacaaggaagccttgcctgccggtacgcagctgcgatgcatccggagcaggtggcaagtgtgacttctgtttcgggtgtcaatttcggcagcgagattgctgagctggttcgccttgctgtggagccgggatccctccccgaagcgctggcgggaactgtcatggacgcggtaggttcattcctttctctgattacaggacatccttgtttgcctcaagattctgtagcagctcttgatgcgctcacctcagaaggcgtagcccgatttaatgcgaagtatccgcaagggctcccaaatacatggggaggagaaggaaaggaagttgaaaacggggtatattattacagctggggcggcataatcaactacaaccctttagatcaaggcctgaacaaccttgacccgcttcacgccgcattggttgctttgtcccttttatttacaaaagaacgctggcagaatgacggcttagtcggtcgttacagcatgcacttagggaaggtcatcagaagtgattattcaatggatcatgcagacgccatcaatcaaacggccgggatggtgacaccggatgctgatccgattacgctgtttgttgagcatgtcgcaagattgaaatcaaaaggcttg

SEQ ID NO: 2 - protein, 294 aa, Serratia sp.
MSTTTKLKYPIILVHGFSGFDKVAGIYPYFYGIEQALEKAGATVFTAAISAENANEVRGEQLLKFVQQVISVTGAEKVNLIGHSQGSLACRYAAAMHPEQVASVTSVSGVNFGSEIAELVRLAVEPGSLPEALAGTVMDAVGSFLSLITGHPCLPQDSVAALDALTSEGVARFNAKYPQGLPNTWGGEGKEVENGVYYYSWGGIINYNPLDQGLNNLDPLHAALVALSLLFTKERWQNDGLVGRYSMHLGKVIRSDYSMDHADAINQTAGMVTPDADPITLFVEHVARLKSKGL

SEQ ID NO: 3 - DNA, 870 bp, Pseudomonas frederiksbergensis
  source 1..870: mol_type = genomic DNA
atgaatatggacgcgtcaacgcaatatccgatagtgcttgttcacggtttgtttggcttcgatacaatcggcggatacccttatttttttgaaatcaaagaagcgcttgaaagggcgggagcaaaagtgtacgctgtcaatattccagcggttaacggcaatgaagagcggggagaaaaactattggagcatgtgaaccgcattcttcgcgaaacaggcgccgccaaggtcaacctgatcggacattcacaaggcccgctggcagcccgatacgtggcagctctgcatccgcaaaaagtagccagtgtcactagtgtgagctgtcccaatcatggatcggaaattgctgatcagcttcataaagcgctgacgcctggcgagctgccagaagcagttgttctggcattattcgccgctgtcggcattttcatctccctaatatccgggcatcctgaaaatccgcaggacgcgcgtgctgcctttgcatcactcacctctgaaggtcttgcggcttttaacaaaaagtatccccagggggttccgaaacattggggtggcgacgggaatgagattgaaaacggagtttattattactcttggtcaggtattgttcagaattttcaatccttacagccactggatccgagccacttaaactgcattgtgctcagtaagctgttttataaagagaaacacgcgaatgacggacttgtcggacaaaacagctctcatttggggaaagtaatcagatctgattatccgatggatcattttgatgctgtaaatcaaatggcagggattacaagctggaatgtctcgcctgtacacctctatttggaacacgcagcaagattaaaggataaaggctta

SEQ ID NO: 4 - protein, 290 aa, Pseudomonas frederiksbergensis
MNMDASTQYPIVLVHGLFGFDTIGGYPYFFEIKEALERAGAKVYAVNIPAVNGNEERGEKLLEHVNRILRETGAAKVNLIGHSQGPLAARYVAALHPQKVASVTSVSCPNHGSEIADQLHKALTPGELPEAVVLALFAAVGIFISLISGHPENPQDARAAFASLTSEGLAAFNKKYPQGVPKHWGGDGNEIENGVYYYSWSGIVQNFQSLQPLDPSHLNCIVLSKLFYKEKHANDGLVGQNSSHLGKVIRSDYPMDHFDAVNQMAGITSWNVSPVHLYLEHAARLKDKGL

SEQ ID NO: 5 - DNA, 882 bp, Enterobacillus tribolii
  source 1..882: mol_type = genomic DNA
atgaaaaaagcaactacgcttaaatatccgattatcttggtgcacggactttttggttttgacaaaatcgctggcgtttatccttattttttcggtgtaaaagaagctcttgaaaaagcgggggcggaagtgtatgtcgcatcactgtcggcagtaaattcaaacgaagttcgcggtgagcagctcatggactttgtcaatgaggtgctggcaaataccggtgcaaagaaggtgaacttgatcggccactctcaaggcccgcttgcctgccgttacgtggctgcattacgccctgatattgttgcttctgtgacaagcgttcatggcgtcaacttcggcagcgagttagccgatgtggtccgtcaggccttgattccagggaggttgcctgaagcgatagctcatgcggtagtcacaacatttggagatttcttatcgctaatttcaggaaagccgatgcttgcgcaggatgcaaaagccgccttagacgcccttacctcagaaggaatcgcagaatttaatgcgaagtacccgcaagggctgccatctgaatggggaggagaaggcgatgaatatgtaaacggcgtatattattacagctggggcggagttttaaaatacaatatctttgatcagctgttgaacaatctggatcccacacatattgcgatgagtgctctttccattttctttaacaaagagcggggacaaaatgacggcgttgtcggtagatactctatgcatttaggaaaagttatacgatctgattattcaatggatcacctcgacgctgtaaatcaaacggcaggggttgtcacgactagtgtcaatccggtgaagctgtatgttgatcatttgtatcttctgagaagcaaaggcctc

SEQ ID NO: 6 - protein, 294 aa, Enterobacillus tribolii
MKKATTLKYPIILVHGLFGFDKIAGVYPYFFGVKEALEKAGAEVYVASLSAVNSNEVRGEQLMDFVNEVLANTGAKKVNLIGHSQGPLACRYVAALRPDIVASVTSVHGVNFGSELADVVRQALIPGRLPEAIAHAVVTTFGDFLSLISGKPMLAQDAKAALDALTSEGIAEFNAKYPQGLPSEWGGEGDEYVNGVYYYSWGGVLKYNIFDQLLNNLDPTHIAMSALSIFFNKERGQNDGVVGRYSMHLGKVIRSDYSMDHLDAVNQTAGVVTTSVNPVKLYVDHLYLLRSKGL

SEQ ID NO: 7 - DNA, 879 bp, Yersinia entomophaga
  source 1..879: mol_type = genomic DNA
atgaaaacgtctacgaagacgcaatatccgattattttagtacacggcctgttcggttttgataaaatgctgggatatccttatttctttaaaattcagccggcgcttgaagtggctggcgcacaggtgtttaccgcctctgtctccgcgacaaacagcaatgaaacaagaggtgaacagctccttgattttatacgttacattttgaataaaacaggtgccaaaaaagtaaacctcatcggacattcacagggccctttagcctgccgctatgctgcagcgatgagaccagatcttgtcgcttcagtgacttccgtaaacggcgtgaatcacggatctgaatttgcggaccgagtaagagaggcgtttgtggaaggcggattgcctgaaagtgtagcaaaccttgtcgtttcgacctttacaaatctgatgtcgctactgtcagggcatcccgagcttccgcaggatgccattgcttctttagacgccttgactacaaaaggtgttactgagtttaatgcaaaatacccgcaaggactgccggaaaaatggggcggagaaggaaaggaagttgaaaacggggtccattattacagctggggaggtttcatccaaggcgggatcctggagcagggcttaaatacggctgatccgcttcatattgcaatgcgcgttggaagccaatttttcatccgtgaggcagaacaaaatgacggcatggtcggccggttcagcatgcatttagggaaagtgataaggtcaaactattcaatggaccacatggatgctgtcaatcaaacagccggtgttgtgcctgttcacctcgatccagtcaagatgtttgttgatcatgcggcatttttaaaaagcaagagtctc

SEQ ID NO: 8 - protein, 293 aa, Yersinia entomophaga
MKTSTKTQYPIILVHGLFGFDKMLGYPYFFKIQPALEVAGAQVFTASVSATNSNETRGEQLLDFIRYILNKTGAKKVNLIGHSQGPLACRYAAAMRPDLVASVTSVNGVNHGSEFADRVREAFVEGGLPESVANLVVSTFTNLMSLLSGHPELPQDAIASLDALTTKGVTEFNAKYPQGLPEKWGGEGKEVENGVHYYSWGGFIQGGILEQGLNTADPLHIAMRVGSQFFIREAEQNDGMVGRFSMHLGKVIRSNYSMDHMDAVNQTAGVVPVHLDPVKMFVDHAAFLKSKSL

SEQ ID NO: 9 - DNA, 864 bp, Arsenophonus nasoniae
  source 1..864: mol_type = genomic DNA
atgccgacaaaatacccaatcattttggtgcacggcctcttcggttttgataaaatcgccggatacccatgctttttcgccattgaaaaccgattaaagaaacaaggctataacgtattttcacccatattatccggtgtaaactcgaatgaagtgaacggcgagcagctttggctgtatatcgaggagttaaaacgcaatatcggctgtgaaaaagtgaatttaatagcccatagtcaaggagcgctgtttgctcgttatgtggcggcaaactattcagcatccattgcaagtgtaactagcatgaatggcgtaaatcacggttctgaaatcgctgatttggtcagaaaagtacttattcctgggaagctgacagaaacggttgtcgttacggctgctgaaatcttttttacatttatttctttaatttcatctggcacgctgaagcctcaggacggcgttgaagcattgaactcgctcaccactgaggttgttaacgaatttaataaaaaatatccgcaagggcttccgaaagaatggcggggagaaggagatgaagttgtgaacggagtgcattattacagcttcggcagctttatcaaaaagtccctgataaacagcggaatcaatgcgtttgacgtgtctcatacatcattactacagctgtcctctttcttcagtagggagaaggaaaatgacggacttgtcggccgctactcaatgagacttggaaaattgatttgcgatgattatgatatggatcatcttgatattgttaatcagattgccggggtcgtcagcaatcaatatgacattccgtcaatttatgtcaatcatgcgcaaatgctggcaaaaaaagggctc

SEQ ID NO: 10 - protein, 288 aa, Arsenophonus nasoniae
MPTKYPIILVHGLFGFDKIAGYPCFFAIENRLKKQGYNVFSPILSGVNSNEVNGEQLWLYIEELKRNIGCEKVNLIAHSQGALFARYVAANYSASIASVTSMNGVNHGSEIADLVRKVLIPGKLTETVVVTAAEIFFTFISLISSGTLKPQDGVEALNSLTTEVVNEFNKKYPQGLPKEWRGEGDEVVNGVHYYSFGSFIKKSLINSGINAFDVSHTSLLQLSSFFSREKENDGLVGRYSMRLGKLICDDYDMDHLDIVNQIAGVVSNQYDIPSIYVNHAQMLAKKGL

SEQ ID NO: 11 - DNA, 882 bp, Yersinia frederiksenii
  source 1..882: mol_type = genomic DNA
atgtctaccaactcgacgttgaaatacccggttgttcttgtgcacggacttttgggttttgataaaatcgccggcatttatccttatttttacggagttgaagagccgctcaaaaaagcaggtgctgatgtgtttattgcgactatatcggctacaaattcaaatgaagtacggggggagcagctactgaaattcatcaaagaagtcatggcgaaaacaggtgcaaaaaaggtgaacctgatcggccattcacagggacccttagcctgccgctatgtggcggctacgcatcctgagctggtcgcatctgtgactagtgtaaacggagtcaaccacggcagcgaaatcgcagacctcgtcagatctgcgctcaccccagacagattacctgaacagatagtgaatacgattatgagtgctttcggggcatttgttagccttctttccggaaagccgtttttgccacaggattttatggaatcaatcaacgccctgacaacagaaaatgtagccaagtttaatacacaatatccgcaagggctgccggaggtttggggaggtgaaggcaaggaatttgacaacggcgtgtactattatagctggggcggctatttaggatataacccattgactgaaggaatgaataaccttgatccgcttcatcactccttggttgcgctttcacttctcttcacaaaagagcgttatcaaaatgacggcatggtcggtaggtacagcatgcatttgggaaaagtcattcgaagtgattataaactggatcatgttgatgcagtcaatcaaacggctgggatggtttcttctgaaattgatcctgtaaagctgtacgtaaatcatattgaattattaaaaagcaaaggctta

SEQ ID NO: 12 - protein, 294 aa, Yersinia frederiksenii
MSTNSTLKYPVVLVHGLLGFDKIAGIYPYFYGVEEPLKKAGADVFIATISATNSNEVRGEQLLKFIKEVMAKTGAKKVNLIGHSQGPLACRYVAATHPELVASVTSVNGVNHGSEIADLVRSALTPDRLPEQIVNTIMSAFGAFVSLLSGKPFLPQDFMESINALTTENVAKFNTQYPQGLPEVWGGEGKEFDNGVYYYSWGGYLGYNPLTEGMNNLDPLHHSLVALSLLFTKERYQNDGMVGRYSMHLGKVIRSDYKLDHVDAVNQTAGMVSSEIDPVKLYVNHIELLKSKGL

SEQ ID NO: 13 - DNA, 870 bp, Pseudomonas sp.
  source 1..870: mol_type = genomic DNA
atggatatggacgcttccactcaatatccgattgtgttgattcatgggctgttcggatttgacaaaatcgccgggtacccatatttctttgacattgaaaacgcgcttgagcgtgcgggtgcgacggtgtttgcggtgaatattccgtctgttcactccaacgaagcgagaggtgaatcattactcgcccatattgaccgcattttactgcagacaggcgcagccagagtcaacctgatcggccacagtcagggaccgctggctgcacgctatgtggcagccctctacccacaaaaggttgccagtgtaacctctgttgcttgcccgaatcatggttcagaaatcgcagatttgcttcaccgggctctgactcccggagaactgcctgaggcacttgtacttgcattactcgggacagtcggcacgctaatagcgttgatatcaggctctcctcagccggttgacccgcaggcggcattcggcagcctaacgacagccggaatggctgattttaacagaaaatatcctcaaggtatgccggctgaatggggaggcgaaggccgtgaaagagaagataatggcgtccattattacagctggtcaggaatcgttcaaaactttcagtcgctgcagcctcttgatccttctcacttaaacagccttgtattaagcaagttttttgtcagggagcggcatgcaaatgatggcttggtaggtcgatactcaagccatttaggaaaagtgatccgttctgattatccgatggatcattttgatgctgttaatcaaatggcgggaattacatcgtggaatgtcaatccagtcgggctctatctggagcatgcggctcggcttcgccaaaaagggttg

SEQ ID NO: 14 - protein, 290 aa, Pseudomonas sp.
MDMDASTQYPIVLIHGLFGFDKIAGYPYFFDIENALERAGATVFAVNIPSVHSNEARGESLLAHIDRILLQTGAARVNLIGHSQGPLAARYVAALYPQKVASVTSVACPNHGSEIADLLHRALTPGELPEALVLALLGTVGTLIALISGSPQPVDPQAAFGSLTTAGMADFNRKYPQGMPAEWGGEGREREDNGVHYYSWSGIVQNFQSLQPLDPSHLNSLVLSKFFVRERHANDGLVGRYSSHLGKVIRSDYPMDHFDAVNQMAGITSWNVNPVGLYLEHAARLRQKGL

SEQ ID NO: 15 - DNA, 867 bp, Pseudomonas sp.
  source 1..867: mol_type = genomic DNA
atgagcaaagaagcgtcgactcaatatccaatggtgctcgttcacgggctcttcggatttgattccatcgccggctatccttattttttcaatattcagccggcacttgagagagccggtgcaaaggtatttacagtgaacattcccgcggtcaacggaaacgaagagcggggtgaaaagctgcttgaacaagtaaacttaatactgcagcaaacgggggcagccaaagtgaatctgatcggacattcacaaggacccctggcagctcgttatgtggctgcgattcatccggaaaaagttgccagtgtcacgtctgtttcctgcccgaatttcggcagtgagattgctgatcagcttcgcaaagcattaattcctggaacgcttccaaccgctgttgctgaagcaatcttaaacgctgtcggcatttttatttctttgatcagcggccatccaacaaatcctcaggatgcggcagcagcatttgaatcattaacaacagaaggccttgccgcttttaacctgaaatacccgcaaggcgttcctgctgtatggggcggagagggcaatgaagtggaaaacggtgtctactattacagctggtcagggatcgttcaggggtcgaagccgcagcttttagatttgagccatttgaactgtattgccctttccttattgttttataatgagaaaaatgcgaatgacggattggtaggccaaaacagctctcaccttggtaaagtcatcaaatcagattatccgatggatcattttgacgcagttaatcaacttgcaggtataactggctggaatgtcaatccggtgcagctgtacttagaccacgcagtgctgctaaagtctaaaggactc

SEQ ID NO: 16 - protein, 289 aa, Pseudomonas sp.
MSKEASTQYPMVLVHGLFGFDSIAGYPYFFNIQPALERAGAKVFTVNIPAVNGNEERGEKLLEQVNLILQQTGAAKVNLIGHSQGPLAARYVAAIHPEKVASVTSVSCPNFGSEIADQLRKALIPGTLPTAVAEAILNAVGIFISLISGHPTNPQDAAAAFESLTTEGLAAFNLKYPQGVPAVWGGEGNEVENGVYYYSWSGIVQGSKPQLLDLSHLNCIALSLLFYNEKNANDGLVGQNSSHLGKVIKSDYPMDHFDAVNQLAGITGWNVNPVQLYLDHAVLLKSKGL

SEQ ID NO: 17 - DNA, 897 bp, Snodgrassella alvi
  source 1..897: mol_type = genomic DNA
atgttgaacatcatcaaacctaacaaaatcgttaaaacccgctatcctattgtcctggtccatggcatattcggatttgatcgtatcatgggatatccttacttcttcaaaattgcagactcattaagaaagctgggctgtgaagtatacacaccagcagtaagtgcgacaaacacaacagaagaacgcggcaaacagcttcttgcagaagttcgaaagatcctccgtaagtcaggagctgagaaagtgaatttaattggacatagccagggttccccgacctgccggtacgtagcggccctccacccggaacttgtcggctccgtcactagtgtcaatggcgtgaattttggttccgagattgcggacctaatgcttgacattctgagcggcaaacttgtgggcaattctgcaaacctgatcgtggaatcgtttatgaagctcatttcactattgtcgacgaagccgctgctgccgcaggattttaagggcagcttaaaaagcttatcaactgaaggaacgaacgagtttaataaacaatatccacaagggctgcctgaaacatggggcggacagggaaaagagcttgagacgaatggagtttattattattcttggtctggtattataaaactgaacgctgttaatgaaggactcaatattttggatcccacgcacgcgattttagttgcactgtcagctttttttaaaaaagaaaggaaacaaaatgatggtctagttgggcggtacgccactcatttggggaaagtcatcggctctgattatcaaatggaccacttagatgcgataaaccaagtggctggtgcccatccgacaaaattggatccggtaaagctttatcttgatcatgccgctagacttcattttaaagggctc

SEQ ID NO: 18 - protein, 299 aa, Snodgrassella alvi
MLNIIKPNKIVKTRYPIVLVHGIFGFDRIMGYPYFFKIADSLRKLGCEVYTPAVSATNTTEERGKQLLAEVRKILRKSGAEKVNLIGHSQGSPTCRYVAALHPELVGSVTSVNGVNFGSEIADLMLDILSGKLVGNSANLIVESFMKLISLLSTKPLLPQDFKGSLKSLSTEGTNEFNKQYPQGLPETWGGQGKELETNGVYYYSWSGIIKLNAVNEGLNILDPTHAILVALSAFFKKERKQNDGLVGRYATHLGKVIGSDYQMDHLDAINQVAGAHPTKLDPVKLYLDHAARLHFKGL

SEQ ID NO: 19 - DNA, 867 bp, Buttiauxella brennerae
  source 1..867: mol_type = genomic DNA
atgtgcacaaaatacccagtcgttctcgttcatggctggagcggcttttctacgattcttggctatccatattatttcggtgtgaaggaagcgcttgagaagaagggagcagatgtgtatacggcgtctttgtccggagtcaatacagacgatgtcagaggtgaacagctgtgggattttattcaggatgtaaagcgaaaaagcggcaaagataaagtgaacctgatcggccattcacaaggcgcgttggactgtcggtatgtggctgctgtttatccgcattctgtcgcttcagtaactagcgttgatggcgcaaatcacggctcagagtccgctgatgcgcttagagcagcctatgaaccggggtcttgcaaagaaggatttgtcgcgctagcagtgaatgcatttgaaaaagccatcgccttcctttcgggacatccgtttgagcccgaagactttatcgcttctttaaattccctgacgacagaaggggtacaggcgtttaacgaaaaatatcctcaaggtctccctgaagtgtggggaggagaaggccctgaggttgtcaacggtatttattactacagctggagtggcattataaaagacgggatatgcgaacaaggattgaatgagctggatccgcttcacttatggatgaaacatggggccaaaacatttgtgaatgaagtagatcaaaatgacgggttggtaggtaggtacagttcacacctcggaaaagtgatttgttcagattatagcatggatcatttagatgcaatcaatcagttagccggaatccgtacaaacaccgttaacgttattgatctgtacactgaccatcttgacttcttacgctcgaagggtgtc

SEQ ID NO: 20 - protein, 289 aa, Buttiauxella brennerae
MCTKYPVVLVHGWSGFSTILGYPYYFGVKEALEKKGADVYTASLSGVNTDDVRGEQLWDFIQDVKRKSGKDKVNLIGHSQGALDCRYVAAVYPHSVASVTSVDGANHGSESADALRAAYEPGSCKEGFVALAVNAFEKAIAFLSGHPFEPEDFIASLNSLTTEGVQAFNEKYPQGLPEVWGGEGPEVVNGIYYYSWSGIIKDGICEQGLNELDPLHLWMKHGAKTFVNEVDQNDGLVGRYSSHLGKVICSDYSMDHLDAINQLAGIRTNTVNVIDLYTDHLDFLRSKGV

SEQ ID NO: 21 - DNA, 885 bp, Entomomonas sp.
  source 1..885: mol_type = genomic DNA
atggactcaaaatcaaacaatagtgcgattatcaattcaactaagtacccaattttgcttgtccacgggttgttcggctttgaaaaaattgccggatacccctacttttataaaatagatgagctgctgcgacagcaaggagcgaatgtattcacacctgttgtatcggctgcaaatacaacgaaaaacagaggggaacagcttcttttgcagattaaacaaatccttgatcttactaaagcagacaaagtaaacctcattggccattctcacggagcgcttacggcacgttatgtggcagcctgctacccagagcttgttgcttcagtcacctcggtgaatggtgtaaatcatggttcagaaattgctgacgtgatgttaaaggttctgaagaacaaactttcatcatcaatagccaacaagctgatctctcactttgtcaacagcgttaccctgttatcaacaaagcggcatctgcctcaggattttatcggcgctttgaactgcctgtctactgaaggagttaaacattttaataaccaatatccgcagggcattccgacaacatgggggggagaaggcttagagctcgaaaacaacaatgtgtattattacagctggagcggtatcttaaatacgatcccgattacgctgtcaaataaattctccttactcagtttgagctcccgctattttgtgaaagaacttcaacaaaatgacggcctagtcggccgtttttcctctcatttaggtaaggtcatccgctctgattatccgatggatcatgcagcggcggttaatcagatcaggggaaaatgtaatgcatccattgatcctacagccttatatattgagcatttacaaagattggctctcaaagggcta

SEQ ID NO: 22 - protein, 295 aa, Entomomonas sp.
MDSKSNNSAIINSTKYPILLVHGLFGFEKIAGYPYFYKIDELLRQQGANVFTPVVSAANTTKNRGEQLLLQIKQILDLTKADKVNLIGHSHGALTARYVAACYPELVASVTSVNGVNHGSEIADVMLKVLKNKLSSSIANKLISHFVNSVTLLSTKRHLPQDFIGALNCLSTEGVKHFNNQYPQGIPTTWGGEGLELENNNVYYYSWSGILNTIPITLSNKFSLLSLSSRYFVKELQQNDGLVGRFSSHLGKVIRSDYPMDHAAAVNQIRGKCNASIDPTALYIEHLQRLALKGL

SEQ ID NO: 23 - DNA, 882 bp, Arsenophonus sp.
  source 1..882: mol_type = genomic DNA
atgagcacaaaataccctatcatattggttcacggttttttcggtttcgaccgtattgccggatatccatatttcttctctattgaatcgaggctgcaggaacagggctataacgtctatattccaacgctttccggtgcaaattcaaatgaagttaacggcgagcaattatgggaattcattgatgaaattaaacgcaaggctggctgcgagaaagtaaacctaattgcccactctcaaggcgcgctttatgcgcggtacgtagcagcaaactatccggcgtctatcgcttccgtgactacaatgaatggggtaaattacggaagtgaaatcgcggatttactccgaaaaatcttattgcctggaatgctggcggagcggcttgttacaaccactgctgaagtgttttttaaatttattagtctgctttctagcggaacgctgaaaccgcaggacggcgtgaaggcccttgaaagcctcaccacgaaagtcgtgaacgaatttaataaaaaatacccgcaaggtttaccgacagaatggggaggagaaggcgacgaggttgtcaatggagtttactattattcctacgattcgtttatcaaaaacagcttgcttgatatcggcattaacatgtttgatatttcacatttgcccctcagacagctgaataagctgtttgtgaaagaaaaagagaaagaaaaggagaaggaaaatgatgggcttgtcggacgttattcaatgagactcggcaaattgatccgcgatgactataatatggatcattttgacatcgtgaatcaaatagcagggtttgtctcaaacaaatatgatgttcctcagatttatgtaaatcatgctcaaatattagcaaagagagggctg

SEQ ID NO: 24 - protein, 294 aa, Arsenophonus sp.
MSTKYPIILVHGFFGFDRIAGYPYFFSIESRLQEQGYNVYIPTLSGANSNEVNGEQLWEFIDEIKRKAGCEKVNLIAHSQGALYARYVAANYPASIASVTTMNGVNYGSEIADLLRKILLPGMLAERLVTTTAEVFFKFISLLSSGTLKPQDGVKALESLTTKVVNEFNKKYPQGLPTEWGGEGDEVVNGVYYYSYDSFIKNSLLDIGINMFDISHLPLRQLNKLFVKEKEKEKEKENDGLVGRYSMRLGKLIRDDYNMDHFDIVNQIAGFVSNKYDVPQIYVNHAQILAKRGL

SEQ ID NO: 25 - DNA, 882 bp, Yersinia enterocolitica
  source 1..882: mol_type = genomic DNA
atgagcacgaacagcactttaaaatacccggttgtgttagttcacggcctgcttggttttgataagatcgccggtgtttatccatatttttacggcgttgaagaacctttgaaaaaagcgggcgcacaggtgtttgtcgcaaccatctccgctacaaactcaaatgaagtaagaggcgaacagcttttgaagtttgtgaaagaagtcatggcaaaaacaggagccaagaaagtgaacttgatcggccacagccaaggcccgctagcttgccgatatgtggcggcgactcatccggagcttattgcatctgtaacgtcagtaaacggggtcaatcacgggagtgagattgctgaccttgtcagatcggctttggtcccaggatcactccccgagcatattgtgaatacaattatgagtgctttcggagtattcgtttctcttttatccggaaaaccgttcctgcctcaggattttatggaaagcatcgacgcgctgaccacagaaaatgtcgcgaaatttaacacgaaatatccgcagggtcttcctgaaacgtgggggggcgaggggaaagaatttgacaatggcgtatattattacagctggggaggtgtccttggctataacccgctcattgaaggcttaaataatctggatccactccatcattctctcgtggccttatcgctgctgttcacaaaagaacgcaaccaaaatgacgggttagtcggtcggtactccatgcatttaggtaaagtcatacgttcagattatcaacttgatcatgttgatgccatcaatcaaacagcaggaatggtttcaaaggatatagatcctgttcaattatttgttaatcagattgaattgctgaagtctaaaggactg

SEQ ID NO: 26 - protein, 294 aa, Yersinia enterocolitica
MSTNSTLKYPVVLVHGLLGFDKIAGVYPYFYGVEEPLKKAGAQVFVATISATNSNEVRGEQLLKFVKEVMAKTGAKKVNLIGHSQGPLACRYVAATHPELIASVTSVNGVNHGSEIADLVRSALVPGSLPEHIVNTIMSAFGVFVSLLSGKPFLPQDFMESIDALTTENVAKFNTKYPQGLPETWGGEGKEFDNGVYYYSWGGVLGYNPLIEGLNNLDPLHHSLVALSLLFTKERNQNDGLVGRYSMHLGKVIRSDYQLDHVDAINQTAGMVSKDIDPVQLFVNQIELLKSKGL

SEQ ID NO: 27 - DNA, 876 bp, Yersinia massiliensis
  source 1..876: mol_type = genomic DNA
atgagctcatctctcaagtatccgattatacttgttcacggcttcagcggatttgataaaattgcgggtatttacccttattttttcggcattcagcaggcgcttgaaaaagcaggtgcaaccgtttttactgcgtcaatatcagctgaaaacagcaatgaagcaagaggagagcagttgctgtcctttgtgaaacaagtaacacagcttaccggggctcataaagtgaacctgatcggacactctcaaggcccactggcctgccgttatgtggctgcgattcacccggaaagagtcgcatccgtaacgtctgtcaatggagcaaattttggaagtgaaatcgctgaccttgtacggttagcgatgacacccggttctttacctgaagtcattgccggcgctgtcatgaatgctttcggaacgtttttgtccatcatgacgggccgtccttcattgccgcaggattctgtagcggctttaaattcattgactagtgaaggcgtcgcaaaatttaatgcgaaatatcctcaagggctgccaagtaactggggcgaagagggaaaagagtatgttaacggtgtttattattacagctggggaggggtgattaactacaatccaattgaacaaggattaaacaactttgacccgcttcatacatcgatggttgccctatcgttcctttttactaaagaacgcctgcaaaatgacggccttgtcggccgatactcaatgcatctgggcaaggtgatccgctccgattatagcatggatcatttagatgcaatcaatcaaacagccggtgccgtcacaacgagcacagatccggttcagctatttgttgagcatgtggcgaggctggcatctaaggggctc

SEQ ID NO: 28 - protein, 292 aa, Yersinia massiliensis
MSSSLKYPIILVHGFSGFDKIAGIYPYFFGIQQALEKAGATVFTASISAENSNEARGEQLLSFVKQVTQLTGAHKVNLIGHSQGPLACRYVAAIHPERVASVTSVNGANFGSEIADLVRLAMTPGSLPEVIAGAVMNAFGTFLSIMTGRPSLPQDSVAALNSLTSEGVAKFNAKYPQGLPSNWGEEGKEYVNGVYYYSWGGVINYNPIEQGLNNFDPLHTSMVALSFLFTKERLQNDGLVGRYSMHLGKVIRSDYSMDHLDAINQTAGAVTTSTDPVQLFVEHVARLASKGL

SEQ ID NO: 29 - DNA, 882 bp, Escherichia sp.
  source 1..882: mol_type = genomic DNA
atgaagattcagacgcaattaaattaccctgtcgtgcttgtccacggcttgttcggttttgataaaattgcaggggtttatccgtatttttacggcatcaaagatgccttggaagaagctggggccaccgtgttcatcgcttctatttcagcagtaaatgacaatgagcttcggggagagcagctgcttgcatatatcaatgatgtgctgaaaaaaacaggaaaagagaaggttaacctcatcggccattcacaggggcctttggcttgccgctatgtggctgcaacacaccccacattagttgcctctgtcacttctgtaaacggtgtgaatttcggctcagagttcgcggacctcgttagatctgcgctcattccgggtgaaatccctgaagtcattgccaacagtatacttgacgtttttgcgaagctgctgacggccatctccggaaatccggattttccgcaggattcgatagctgcgctggatgcgctaacaacggaaggggtagcaaaatttaacgaaaaatatcctcaaggactcccgattgtacgcggcggtgaaggcaaagaatttgacaacggtgtatattattacagctggagcggcattatagacagcaatatcctgcatcaaggcatgaataactttgatccatctcatattgcgatgctcgcttgtagcatgctgtttgaaaatgaatatcatgaaaacgacggacttgtcggccgttatgcgtcccacttaggaaaggttatcagaagcgattattcgcttgatcatttggatgcaattaatcaaattgcaggagtgttgccacgatacagtgattcaatctccatttaccttgagcatttagagaggttaaaatcaaaaggatta

SEQ ID NO: 30 - protein, 294 aa, Escherichia sp.
MKIQTQLNYPVVLVHGLFGFDKIAGVYPYFYGIKDALEEAGATVFIASISAVNDNELRGEQLLAYINDVLKKTGKEKVNLIGHSQGPLACRYVAATHPTLVASVTSVNGVNFGSEFADLVRSALIPGEIPEVIANSILDVFAKLLTAISGNPDFPQDSIAALDALTTEGVAKFNEKYPQGLPIVRGGEGKEFDNGVYYYSWSGIIDSNILHQGMNNFDPSHIAMLACSMLFENEYHENDGLVGRYASHLGKVIRSDYSLDHLDAINQIAGVLPRYSDSISIYLEHLERLKSKGL

SEQ ID NO: 31 - DNA, 882 bp, Mixta intestinalis
  source 1..882: mol_type = genomic DNA
atgagcaaagtgacaaagctgaaatatccagtcattttggttccttctttgttcggctttgagaaaatcgccggaatttatccgctgttttatggtgttcaaaaagtattagaaaaagcaggtgccgttgtttttactgcgccgattagcgtagaaaattcaaatgaagtgcgcggagaacagctgatagcaagcatccgcgatgtcatcaaaaaaacaggtgcaaaaaaggtaaacttaatcggctatagccaggggccgcttgcgtgtcgatacgctgccgcaaagcatccggagcttgttgcttctgtaacaagcatttgcggtgccaattacggatcagaatttgctgatctcgtcagggcagcgatcaaaccgggcggccttcctgaactgatcgcttcaacagtcatggacgctttcggaaaatttatgtcggccattaccggaaatccgggtttgccgcagtcatccatagcagctctagactcgctaacgacgaaaggcgtagcggcatttaatgcgaagtatcctcaaggactgccggcggtgtggggcggggacggaccagaggttgtgaacggcgtgtattattactcctggtctggggtcattaactacaaccctttcacccagggatttaacaaccttgatcccgctcacattgcccttgtggcgactagtcttttattcacaaaagaacgttttcaaaatgacggcttagtcggaagatacgcatcccacctcggcaaggtgatcagaagtgattataatatggatcatttggatgctgttaatcaaacgatgggcattgtttctagtgaagcgaaaccattaaaaatttttgaagagcacatggaacggctcaagtcaaaagggctg

SEQ ID NO: 32 - protein, 294 aa, Mixta intestinalis
MSKVTKLKYPVILVPSLFGFEKIAGIYPLFYGVQKVLEKAGAVVFTAPISVENSNEVRGEQLIASIRDVIKKTGAKKVNLIGYSQGPLACRYAAAKHPELVASVTSICGANYGSEFADLVRAAIKPGGLPELIASTVMDAFGKFMSAITGNPGLPQSSIAALDSLTTKGVAAFNAKYPQGLPAVWGGDGPEVVNGVYYYSWSGVINYNPFTQGFNNLDPAHIALVATSLLFTKERFQNDGLVGRYASHLGKVIRSDYNMDHLDAVNQTMGIVSSEAKPLKIFEEHMERLKSKGL

SEQ ID NO: 33 - DNA, 879 bp, Pseudomonas abietaniphila
  source 1..879: mol_type = genomic DNA
atgtatacagaagtcacaacaaaatacccgcttgtgcttgttcacggactgttcggctttgaaagaatcggcgaatttgacatgtttcatggcattgtctccgcccttgaaaaagcaggctgccgtgtccacgtaccagccgtttcaggtgtccatgataacgaaacgcgcggagaacagctgttagagcagattgaacggttcttaaatagaaccggttatctgaaagtaaacctaatcggacacagccaaggggcattaacggcgcgctatgcggcagcgacacgcccagattgggtggcttctgtcacatctgtttcagggccgaatcatggaagtgaggtagctgaccgagtgagaagagctttttcgccgggggaacttcctgagcgtgtagcgtcccgtctaactttgggttttgcccattttctcgccttgctgggcggccgaccagctttaccccaagacccgctgctcgcgcttgatgcgctcaccactgaaggtgtggcccgttttaaccgggcttaccctcaggggttgcctctggaatggggaggtgaaggtgcagagagggtgaacggagtacattattattcatggagcggctgtattcaatccagtttaataaatgagggaagaaatgcctttgatcctcttcacttggcacttcggagctacgcgcgcctgtttgagcgtgaaacggcatttaatgacgggcttgtcggcaggttctcatctcatttaggaaaagtgatccgatctgattatccgatggatcatgttgatacaatcaatcaaacggcaggcgttgttcgcaagagcattgatccggttaagctgtatattgaccatgctggcttactcttcagaaaaggactg

SEQ ID NO: 34 - protein, 293 aa, Pseudomonas abietaniphila
MYTEVTTKYPLVLVHGLFGFERIGEFDMFHGIVSALEKAGCRVHVPAVSGVHDNETRGEQLLEQIERFLNRTGYLKVNLIGHSQGALTARYAAATRPDWVASVTSVSGPNHGSEVADRVRRAFSPGELPERVASRLTLGFAHFLALLGGRPALPQDPLLALDALTTEGVARFNRAYPQGLPLEWGGEGAERVNGVHYYSWSGCIQSSLINEGRNAFDPLHLALRSYARLFERETAFNDGLVGRFSSHLGKVIRSDYPMDHVDTINQTAGVVRKSIDPVKLYIDHAGLLFRKGL